European Patent Application EP 4 464 774 A1, published November 20, 2024. Title: Cell culture scaffold and method for manufacturing thereof. Applicant: Amolifescience. The sequence listing filed with the application follows.

SEQUENCE LISTING (29 sequences)

SEQ ID NO: 1 - protein, 10 aa, Artificial Sequence
AKPSYPPTYK

SEQ ID NO: 2 - protein, 20 aa, Artificial Sequence
AKPSYPPTYKAKPSYPPTYK

SEQ ID NO: 3 - protein, 60 aa, Artificial Sequence
AKPSYPPTYKAKPSYPPTYKAKPSYPPTYKAKPSYPPTYKAKPSYPPTYKAKPSYPPTYK

SEQ ID NO: 4 - protein, 39 aa, Artificial Sequence
EVHACKPNPCKNNGRCYPDGKTGYKCKCVGGYSGPTCAC

SEQ ID NO: 5 - protein, 52 aa, Artificial Sequence
ADYYGPKYGPPRRYGGGNYNRYGGSRRYGGYKGWNNGWKRGRWGRKYYEFEF

SEQ ID NO: 6 - protein, 46 aa, Artificial Sequence
ADYYGPKYGPPRRYGGGNYNRYGRRYGGYKGWNNGWKRGRWGRKYY

SEQ ID NO: 7 - protein, 60 aa, Artificial Sequence
GHVHRHRVLHKHVHNHRVLHKHLHKHQVLHGHVHRHQVLHKHVHNHRVLHKHLHKHQVLH

SEQ ID NO: 8 - protein, 75 aa, Artificial Sequence
SSEEYKGGYYPGNAYHYHSGGSYHGSGYHGGYKGKYYGKAKKYYYKYKNSGKYKYLKKARKYHRKGYKKYYGGSS

SEQ ID NO: 9 - protein, 76 aa, Artificial Sequence
SSEEYKGGYYPGNTYHYHSGGSYHGSGYHGGYKGKYYGKAKKYYYKYKNSGKYKYLKKARKYHRKGYKKYYGGGSS

SEQ ID NO: 10 - protein, 71 aa, Artificial Sequence
YDDYSDGYYPGSAYNYPSGSHWHGHGYKGKYYGKGKKYYYKFKRTGKYKYLKKARKYHRKGYKKHYGGSSS

SEQ ID NO: 11 - protein, 76 aa, Artificial Sequence; identical to SEQ ID NO: 9

SEQ ID NO: 12 - protein, 99 aa, Artificial Sequence
GGGNYRGYCSNKGCRSGYIFYDNRGFCKYGSSSYKYDCGNYAGCCLPRNPYGRVKYYCTKKYSCPDDFYYYNNKGYYYYNDKDYFNCGSYNGCCLRSGY

SEQ ID NO: 13 - protein, 194 aa, Artificial Sequence
AKPSYPPTYKAKPSYPPTYKAKPSYPPTYKAKPSYPPTYKAKPSYPPTYKAKPSYPPTYKSSEEYKGGYYPGNAYHYHSGGSYHGSGYHGGYKGKYYGKAKKYYYKYKNSGKYKYLKKARKYHRKGYKYYGGSSAKPSYPPTYKAKPSYPPTYKAKPSYPPTYKAKPSYPPTYKAKPSYPPTYKAKPSYPPTYK

SEQ ID NO: 14 - protein, 196 aa, Artificial Sequence
AKPSYPPTYKAKPSYPPTYKAKPSYPPTYKAKPSYPPTYKAKPSYPPTYKAKPSYPPTYKSSEEYKGGYYPGNTYHYHSGGSYHGSGYHGGYKGKYYGKAKKYYYKYKNSGKYKYLKKARKYHRKGYKKYYGGGSSAKPSYPPTYKAKPSYPPTYKAKPSYPPTYKAKPSYPPTYKAKPSYPPTYKAKPSYPPTYK

SEQ ID NO: 15 - protein, 60 aa, Artificial Sequence; identical to SEQ ID NO: 3

SEQ ID NO: 16 - protein, 16 aa, Artificial Sequence
KGGPQCVTRGDVFCTP

SEQ ID NO: 17 - protein, 10 aa, Artificial Sequence
GACRGDCLGA

SEQ ID NO: 18 - protein, 12 aa, Artificial Sequence
SETQRGDVFVPM

SEQ ID NO: 19 - protein, 12 aa, Artificial Sequence
PMQKMRGDVFSP

SEQ ID NO: 20 - protein, 10 aa, Artificial Sequence
EAPRGDVYQG

SEQ ID NO: 21 - protein, 14 aa, Artificial Sequence
SECTQRGDVFCVPM

SEQ ID NO: 22 - protein, 14 aa, Artificial Sequence
PMQCKMRGDVFCSP

SEQ ID NO: 23 - protein, 12 aa, Artificial Sequence
ECAPRGDVYCQG

SEQ ID NO: 24 - protein, 14 aa, Artificial Sequence
GPQCVTRGDVFCTP

SEQ ID NO: 25 - protein, 16 aa, Artificial Sequence
GGGPQCVTRGDVFCTP

SEQ ID NO: 26 - protein, 6 aa, Artificial Sequence
GRGDSP

SEQ ID NO: 27 - protein, 23 aa, Artificial Sequence
KSSPHSRNSGSGSGSGSGRGDSP

SEQ ID NO: 28 - protein, 90 aa, Artificial Sequence
GPQCVTRGDVFCTPAKPSYPPTYKAKPSYPPTYKAKPSYPPTYKAKPSYPPTYKAKPSYPPTYKAKPSYPPTYKGGGPQCVTRGDVFCTP

SEQ ID NO: 29 - protein, 216 aa, Artificial Sequence
HHHHHHAKPSYPPTYKAKPSYPPTYKAKPSYPPTYKAKPSYPPTYKAKPSYPPTYKAKPSYPPTYKSSEEYKGGYYPGNAYHYHSGGSYHGSGYHGGYKGKYYGKAKKYYYKYKNSGKYKYLKKARKYHRKGYKYYGGSSAKPSYPPTYKAKPSYPPTYKAKPSYPPTYKAKPSYPPTYKAKPSYPPTYKAKPSYPPTYKKGGPQCVTRGDVFCTP